European Patent Application EP 4 692 117 A1, published February 11, 2026. Title: Novel OX40 nanobodies. Applicant: Eberhard Karls Universitaet Tuebingen. The sequence listing filed with the application follows.

SEQUENCE LISTING (38 sequences)

SEQ ID NO: 1 - protein, 8 aa, synthetic construct
SGFTLDNY

SEQ ID NO: 2 - protein, 12 aa, synthetic construct
ISSSGESTNYAD

SEQ ID NO: 3 - protein, 20 aa, synthetic construct
VDDIGTTVQFMCNMGPYEYD

SEQ ID NO: 4 - protein, 8 aa, synthetic construct
SGFTLEDY

SEQ ID NO: 5 - protein, 12 aa, synthetic construct
ISGSGGIRNVAD

SEQ ID NO: 6 - protein, 18 aa, synthetic construct
GFETSYSYSYYCGVHEYD

SEQ ID NO: 7 - protein, 9 aa, synthetic construct
STDTFSMSA

SEQ ID NO: 8 - protein, 11 aa, synthetic construct
ILSDGSTYYAD

SEQ ID NO: 9 - protein, 12 aa, synthetic construct
LRGRLWSNHKDD

SEQ ID NO: 10 - protein, 130 aa, synthetic construct
DVQLQESGGGLVQPGGSLRLSCAASGFTLDNYAIGWFRQAPGKEREGVSCISSSGESTNYADSVKGRFTISRDNAKNTVYLQTNSLKPEDTAVYYCAAVDDIGTTVQFMCNMGPYEYDYWGQGSPVTVSS

SEQ ID NO: 11 - protein, 128 aa, synthetic construct
QVQLVESGGGLVQPGGSLRLSCAASGFTLEDYVIGWFRQAPGKEREEVSCISGSGGIRNVADSMEGRATISRDNAKNTVYLQMNSLKPEDTAVYYCAAGFETSYSYSYYCGVHEYDYWGQGTLVTVSS

SEQ ID NO: 12 - protein, 122 aa, unidentified
QVQLQESGGGLVQPGGSLRLSCAGSTDTFSMSAAVSWARQAPGKGLEWVSSILSDGSTYYADSVRGRFTISRDNANNTGSLQMNNLKVEDTAVYYCTNLRGRLWSNHKDDYGGQGSRVTVSS

SEQ ID NO: 13 - protein, 8 aa, synthetic construct
SGFTFGSY

SEQ ID NO: 14 - protein, 11 aa, synthetic construct
IYSDGSTYYAD

SEQ ID NO: 15 - protein, 8 aa, synthetic construct
WGAAAPYD

SEQ ID NO: 16 - protein, 117 aa, synthetic construct
DVQLVESGGGLVQPGGSLRLSCAASGFTFGSYAMGWARQVPGKGLEWVSGIYSDGSTYYADSVKGRFTISRDNAKNTVYLQMNSLKPEDTAVYYCATWGAAAPYDYWGQGTQVTVSS

SEQ ID NO: 17 - DNA, 23 bp, synthetic construct
  source 1..23: mol_type = other DNA
gtcctggctgctcttctacaagg

SEQ ID NO: 18 - DNA, 23 bp, synthetic construct
  source 1..23: mol_type = other DNA
ggtacgtgctgttgaactgttcc

SEQ ID NO: 19 - DNA, 33 bp, synthetic construct
  source 1..33: mol_type = other DNA
catggcnsangtgcagctggtggantcnggngg

SEQ ID NO: 20 - DNA, 33 bp, synthetic construct
  source 1..33: mol_type = other DNA
catggcnsangtgcagctgcaggantcnggngg

SEQ ID NO: 21 - DNA, 33 bp, synthetic construct
  source 1..33: mol_type = other DNA
catggcnsangtgcagctggtgganagyggngg

SEQ ID NO: 22 - DNA, 33 bp, synthetic construct
  source 1..33: mol_type = other DNA
catggcnsangtgcagctgcagganagyggngg

SEQ ID NO: 23 - DNA, 38 bp, synthetic construct
  source 1..38: mol_type = other DNA
gtaggcccagccggccatggcnsangtgcagctggtgg

SEQ ID NO: 24 - DNA, 39 bp, synthetic construct
  source 1..39: mol_type = other DNA
gtaggcccagccggccatggcnsangtgcagctgcagga

SEQ ID NO: 25 - DNA, 35 bp, synthetic construct
  source 1..35: mol_type = other DNA
gatgcggccgcnganganacggtgaccngnryncc

SEQ ID NO: 26 - DNA, 35 bp, synthetic construct
  source 1..35: mol_type = other DNA
gatgcggccgcnganganacggtgaccngngancc

SEQ ID NO: 27 - DNA, 35 bp, synthetic construct
  source 1..35: mol_type = other DNA
gatgcggccgcnganganacggtgaccngrctncc

SEQ ID NO: 28 - DNA, 35 bp, synthetic construct
  source 1..35: mol_type = other DNA
gatgcggccgcrctnganacggtgaccngnryncc

SEQ ID NO: 29 - DNA, 35 bp, synthetic construct
  source 1..35: mol_type = other DNA
gatgcggccgcrctnganacggtgaccngngancc

SEQ ID NO: 30 - DNA, 35 bp, synthetic construct
  source 1..35: mol_type = other DNA
gatgcggccgcrctnganacggtgaccngrctncc

SEQ ID NO: 31 - DNA, 20 bp, synthetic construct
  source 1..20: mol_type = other DNA
cagtacatcaatgggcgtgg

SEQ ID NO: 32 - DNA, 43 bp, synthetic construct
  source 1..43: mol_type = other DNA
gagagactgcacgcacgcgatccggcatggtggcgctagccag

SEQ ID NO: 33 - DNA, 41 bp, synthetic construct
  source 1..41: mol_type = other DNA
cgtgcgtgcagtctctcactggagcagcccgtgcgggccgg

SEQ ID NO: 34 - DNA, 21 bp, synthetic construct
  source 1..21: mol_type = other DNA
gcggaattctcagatcttggc

SEQ ID NO: 35 - DNA, 18 bp, synthetic construct
  source 1..18: mol_type = other DNA
gggagacccaagctggct

SEQ ID NO: 36 - DNA, 30 bp, synthetic construct
  source 1..30: mol_type = other DNA
ggctgctccagtgagagactgcacgcacgc

SEQ ID NO: 37 - DNA, 48 bp, synthetic construct
  source 1..48: mol_type = other DNA
gcagtctctcactggagcagccgatgtcgagctggcacccagcccctg

SEQ ID NO: 38 - DNA, 46 bp, synthetic construct
  source 1..46: mol_type = other DNA
gcagtctctcactggagcagcccttgtcctccagggcacttctccc